European Patent Specification EP 3 750 984 B1, published August 12, 2026. Title: TRANSFORMED, SALMO SALAR INTERFERON GAMMA (IFNG)-PRODUCING LACTOCOCCUS LACTIS BACTERIUM,. Applicant: CONSORCIO TECNOLOGICO DE SANIDAD ACUICOLA S.A. (90%) UNIVERSIDAD DE SANTIAGO DE CHILE (10%). The sequence listing filed with the application follows.

SEQUENCE LISTING (27 sequences)

SEQ ID NO: 1 - DNA, 779 bp, Artificial Sequence
  gene encoding to Salmo Salar immunostimulating protein
ccatggtatagatctaattaatctataaaccatatccctctttggaatcaaaatttattatctactcctttgtagatatgttataatacaagtatcaatgatctgggagaccacaacggtttcccactagaaataattttgtttaactttagaaaggagatatacgcatgaaaaaaaagattatctcagctattttaatgtctacagtgatactttctgctgcagccccgttgtcaggtgtttacgctgctcaatatacatcaattaatatgaaatcaaatattgataaacttaaagtacattataaaattagtaaagatcaattgtttaatggaaaaccagtttttcctaaagatacatttgaagattcagaacgtagagtttggatgtctgttgtattagatgtatatcgttcaatttttaatcaaatgcttaatcaaacaggtgatcaagaagtacgtgaaagattagatcaagttaaaggaaaagtacaagaaactcaaaaacattattttcttaaacgaattccagaattgagaacacatttgcaaaatctttgggctattgaaactagtaatacaactgttcaaggaaaagcattgtcagaatttattactatttatgaaaaagcttctaaattagcacttaaaattcatttaaagaaagataatcgacgtaaaagacgacaagcacaacgattgaaaagtagtattatgggaggtggacatcatcatcatcatcattaaaaaaaagtcttaaaataataaaaatagtctaga

SEQ ID NO: 2 - DNA, 161 bp, Artificial Sequence
  Primer P1, L. lactis; Primer expressing IFNg
tatagatctaattaatctataaaccatatccctctttggaatcaaaatttattatctactcctttgtagatatgttataatacaagtatcaatgatctgggagaccacaacggtttcccactagaaataattttgtttaactttagaaaggagatatacgc

SEQ ID NO: 3 - DNA, 81 bp, Artificial Sequence
  Usp45, secreting IFNg
atgaaaaaaaagattatctcagctattttaatgtctacagtgatactttctgctgcagccccgttgtcaggtgtttacgct

SEQ ID NO: 4 - DNA, 468 bp, Artificial Sequence
  IFNg precursor
gctcaatatacatcaattaatatgaaatcaaatattgataaacttaaagtacattataaaattagtaaagatcaattgtttaatggaaaaccagtttttcctaaagatacatttgaagattcagaacgtagagtttggatgtctgttgtattagatgtatatcgttcaatttttaatcaaatgcttaatcaaacaggtgatcaagaagtacgtgaaagattagatcaagttaaaggaaaagtacaagaaactcaaaaacattattttcttaaacgaattccagaattgagaacacatttgcaaaatctttgggctattgaaactagtaatacaactgttcaaggaaaagcattgtcagaatttattactatttatgaaaaagcttctaaattagcacttaaaattcatttaaagaaagataatcgacgtaaaagacgacaagcacaacgattgaaaagtagtattatg

SEQ ID NO: 5 - DNA, 24 bp, Artificial Sequence
  nucleotide sequence encoding an amino acid terminal sequence
ggaggtggacatcatcatcatcat

SEQ ID NO: 6 - DNA, 20 bp, Artificial Sequence
  FW primer IFNg salmon
ccgtacaccgattgaggact

SEQ ID NO: 7 - DNA, 20 bp, Artificial Sequence
  RV primer IFNg salmon
gcggcattactccatcctaa

SEQ ID NO: 8 - DNA, 20 bp, Artificial Sequence
  FW primer IL1b salmon
ccccattgagactaaagcca

SEQ ID NO: 9 - DNA, 20 bp, Artificial Sequence
  RV primer IL1b salmon
gcaacctcctctaggtgcag

SEQ ID NO: 10 - DNA, 20 bp, Artificial Sequence
  FW primer TGF-B salmon
agctctcggaagaaacgaca

SEQ ID NO: 11 - DNA, 20 bp, Artificial Sequence
  RV primer TGF-B salmon
agtagccagtgggttcatgg

SEQ ID NO: 12 - DNA, 22 bp, Artificial Sequence
  FW primer gamma IP10 salmon
gtgtctgaatccagaggctcca

SEQ ID NO: 13 - DNA, 22 bp, Artificial Sequence
  RV primer gamma IP10 salmon
tctcatggtgctctctgttcca

SEQ ID NO: 14 - DNA, 23 bp, Artificial Sequence
  FW primer IFNg Lactis-IFNg
cacatttgcaaaatctttgggct

SEQ ID NO: 15 - DNA, 21 bp, Artificial Sequence
  RV primer IFNg Lactis-IFNg
caatcgttgtgcttgtcgtct

SEQ ID NO: 16 - DNA, 21 bp, Artificial Sequence
  FW primer IL-6 salmon
ccttgcggaaccaacagtttg

SEQ ID NO: 17 - DNA, 22 bp, Artificial Sequence
  RV primer IL-6 salmon
cctcagcaaccttcatctggtc

SEQ ID NO: 18 - DNA, 23 bp, Artificial Sequence
  FW primer IL-12 salmon
tgacgctttttctcaccggttgt

SEQ ID NO: 19 - DNA, 22 bp, Artificial Sequence
  RV primer IL-12 salmon
acgctttgcagcatgagcttga

SEQ ID NO: 20 - DNA, 20 bp, Artificial Sequence
  FW primer eF1a salmon
gggtgagtttgaggctggta

SEQ ID NO: 21 - DNA, 20 bp, Artificial Sequence
  RV primer eF1a salmon
ttctggatctcctcaaaccg

SEQ ID NO: 22 - DNA, 30 bp, Artificial Sequence
  FW primer RpoS F. pyschrophilum
gaagatggagaaggtaatttagttgatatt

SEQ ID NO: 23 - DNA, 30 bp, Artificial Sequence
  RV primer RpoS F. pyschrophilum
caaataacatctcctttttctacaacttga

SEQ ID NO: 24 - DNA, 24 bp, Artificial Sequence
  FW primer STAT1
gaccagcgaacccaagaacctgaa

SEQ ID NO: 25 - DNA, 23 bp, Artificial Sequence
  RV primer STAT1
cacaaagcccaggatgcaaccat

SEQ ID NO: 26 - DNA, 19 bp, Artificial Sequence
  FW primer rDNA 16S P. salmonis
agggagactgccggtgata

SEQ ID NO: 27 - DNA, 19 bp, Artificial Sequence
  RV primer rDNA 16S P. salmonis
actacgaggcgctttctca